European Patent Specification EP 3 890 759 B1, published August 23, 2023. Title: IMMUNOSTIMULANT FOR USE AGAINST PATHOGENS. Applicant: SABIOTEC SPIN-OFF SL NEIKER-Instituto Vasco de Investigación y Desarrollo Agrario, S.A. The sequence listing filed with the application follows.

SEQUENCE LISTING (8 sequences)

SEQ ID NO: 1 - DNA, 20 bp, Artificial Sequence
  primer
aargaattggcagttcaatc

SEQ ID NO: 2 - DNA, 25 bp, Artificial Sequence
  primer
gcattttcwattttagcaagtgatg

SEQ ID NO: 3 - DNA, 28 bp, Artificial Sequence
  primer
acatattcagatgcagacagaggttcta

SEQ ID NO: 4 - DNA, 27 bp, Artificial Sequence
  primer
gaaggtgctgtagcaggtgctggctgt

SEQ ID NO: 5 - DNA, 23 bp, Artificial Sequence
  primer
aagcaaatttaggtgctttccaa

SEQ ID NO: 6 - DNA, 20 bp, Artificial Sequence
  primer
gcaatcattgccattgcaga

SEQ ID NO: 7 - DNA, 20 bp, Artificial Sequence
  primer
agagggaaatcgtgcgtgac

SEQ ID NO: 8 - DNA, 21 bp, Artificial Sequence
  primer
caatagtgatgacctggccgt